European Patent Specification EP 3 952 901 B1, published July 2, 2025. Title: Interleukin-4-induced gene 1 (IL4I1) as a biomarker and uses thereof. Applicant: Helmholtz-Zentrum für Umweltforschung GmbH - UFZ. The sequence listing filed with the application follows.

SEQUENCE LISTING (26 sequences)

SEQ ID NO: 1 - DNA, 97 bp, Homo sapiens
tgctgttgacagtgagcgcaggaagaattgttttaggatatagtgaagccacagatgtatatcctaaaacaattcttcctttgcctactgcctcgga

SEQ ID NO: 2 - DNA, 96 bp, Homo sapiens
tgctgttgacagtgagcgaaggcagaagtatgcaaagcattagtgaagccacagatgtaatgctttgcatacttctgcctgtgcctactgcctcgg

SEQ ID NO: 3 - DNA, 21 bp, Homo sapiens
ttccacgatatggatttacgg

SEQ ID NO: 4 - DNA, 21 bp, Homo sapiens
gtttcctgttgcattgagtcc

SEQ ID NO: 5 - DNA, 20 bp, Homo sapiens
ccctcctcaggtggtgtttg

SEQ ID NO: 6 - DNA, 20 bp, Homo sapiens
cgacaaatgaagcagcgtgt

SEQ ID NO: 7 - DNA, 21 bp, Homo sapiens
gacgcctttatcctctctgcg

SEQ ID NO: 8 - DNA, 21 bp, Homo sapiens
acgacctgatccaattctgcc

SEQ ID NO: 9 - DNA, 21 bp, Homo sapiens
ctgaccgcagagtcttttcct

SEQ ID NO: 10 - DNA, 20 bp, Homo sapiens
gagtggtttggctggggtaa

SEQ ID NO: 11 - DNA, 21 bp, Homo sapiens
ctgcctgggtttccatcttct

SEQ ID NO: 12 - DNA, 23 bp, Homo sapiens
gccattcatgtcagagctacact

SEQ ID NO: 13 - DNA, 21 bp, Homo sapiens
ctcgccagtgaaatgatggct

SEQ ID NO: 14 - DNA, 21 bp, Homo sapiens
gtcggagattcgtagctggat

SEQ ID NO: 15 - DNA, 20 bp, Homo sapiens
cgcccgaagacatctaccag

SEQ ID NO: 16 - DNA, 21 bp, Homo sapiens
gatattccaagagcgtgtgcc

SEQ ID NO: 17 - DNA, 26 bp, Homo sapiens
gctaacctttgatgctataactacga

SEQ ID NO: 18 - DNA, 21 bp, Homo sapiens
tttgtgcgcatgtagaatctg

SEQ ID NO: 19 - DNA, 22 bp, Homo sapiens
catcaatgacaaggtggccaag

SEQ ID NO: 20 - DNA, 20 bp, Homo sapiens
gggcttgatggggtgatagg

SEQ ID NO: 21 - DNA, 19 bp, Homo sapiens
gatgggcggcggaaaatag

SEQ ID NO: 22 - DNA, 21 bp, Homo sapiens
gcgtggattctgcataatggt

SEQ ID NO: 23 - DNA, 20 bp, Homo sapiens
acccccatgactccagagaa

SEQ ID NO: 24 - DNA, 21 bp, Homo sapiens
cttgtgcctgcaaaatcgcat

SEQ ID NO: 25 - DNA, 22 bp, Homo sapiens
caccctctagcaatgtcaactc

SEQ ID NO: 26 - DNA, 21 bp, Homo sapiens
cagactcgggatactctctcc